European Patent Application EP 4 361 169 A1, published May 1, 2024. Title: INSECT NEUROPEPTIDES 5. Applicant: SOLASTA Bio Limited. The sequence listing filed with the application follows.

SEQUENCE LISTING (16 sequences)

SEQ ID NO: 1 - protein, 8 aa, synthetic construct
  source 1..8: note = Z peptide
KVKFSAWG

SEQ ID NO: 2 - protein, 8 aa, synthetic construct
  source 1..8: note = SB-P-70
  MOD_RES 8: note = glycinamide
KVKFSAWG

SEQ ID NO: 3 - protein, 11 aa, synthetic construct
  source 1..11: note = SB-P-47
  MOD_RES 11: note = leucinamide
  MOD_RES 1: note = pyroglutamyl-alanine
AIMARPQVPRL

SEQ ID NO: 4 - protein, 8 aa, synthetic construct
  source 1..8: note = SB-P-49
  MOD_RES 8: note = leucinamide
SVPFKPRL

SEQ ID NO: 5 - protein, 19 aa, synthetic construct
  source 1..19: note = SB-P-51
  MOD_RES 19: note = leucinamide
LRQLQSNGEPAYRVRTPRL

SEQ ID NO: 6 - protein, 16 aa, synthetic construct
  source 1..16: note = SB-P-80
  MOD_RES 16: note = leucinamide
NADEDQQQSVDFTPRL

SEQ ID NO: 7 - protein, 10 aa, synthetic construct
  source 1..10: note = SB-P-81
  MOD_RES 10: note = leucinamide
GGSMTFSPRL

SEQ ID NO: 8 - protein, 12 aa, synthetic construct
  source 1..12: note = SB-P-46
  MOD_RES 12: note = leucinamide
SPPYSPPFSPRL

SEQ ID NO: 9 - protein, 10 aa, synthetic construct
  source 1..10: note = SB-P-65
  MOD_RES 10: note = glycinamide
RQKTVFSSWG

SEQ ID NO: 10 - protein, 7 aa, synthetic construct
  source 1..7: note = SB-P-66
  MOD_RES 7: note = glycinamide
PAFSSWG

SEQ ID NO: 11 - protein, 9 aa, synthetic construct
  source 1..9: note = SB-P-86
  MOD_RES 9: note = glycinamide
  MOD_RES 1: note = pyroglutamyl-leucine
LTFTSSWGG

SEQ ID NO: 12 - protein, 8 aa, synthetic construct
  source 1..8: note = SB-P-039
  MOD_RES 1: note = palmitoyl-glutamine
  MOD_RES 8: note = tryptophanamide
QLTFSPDW

SEQ ID NO: 13 - protein, 7 aa, synthetic construct
  source 1..7: note = SB-P-042
  MOD_RES 1: note = pyroglutamyl-leucine
  MOD_RES 7: note = tryptophanamide
LTFSPDW

SEQ ID NO: 14 - protein, 6 aa, synthetic construct
  source 1..6: note = SB-P-69
  MOD_RES 6: note = glycinamide
NFSPWG

SEQ ID NO: 15 - protein, 19 aa, synthetic construct
  source 1..19: note = SB-P-48
  MOD_RES 19: note = leucinamide
EQNVQSNGEPAYRVRTPRL

SEQ ID NO: 16 - protein, 8 aa, synthetic construct
  source 1..8: note = SB-P-41
  MOD_RES 8: note = tryptophanamide
QLTFSPDW